European Patent Application EP 4 328 319 A2, published February 28, 2024. Title: Methods and Compositions for Identifying and Treating Patients with Small Cell LUng Cancer. Applicant: University of Utah Research Foundation. The sequence listing filed with the application follows.

SEQUENCE LISTING (27 sequences)

SEQ ID NO: 1 - DNA, 20 bp, synthetic construct
  misc_feature 1..20: note = Synthetic construct
  source 1..20: mol_type = other DNA
aacttcccgccgccgttgtt

SEQ ID NO: 2 - DNA, 20 bp, synthetic construct
  misc_feature 1..20: note = Synthetic construct
  source 1..20: mol_type = other DNA
caacgggccacaactcctca

SEQ ID NO: 3 - DNA, 22 bp, synthetic construct
  misc_feature 1..22: note = Synthetic construct
  source 1..22: mol_type = other DNA
tggaggaggacaaactggtcac

SEQ ID NO: 4 - DNA, 22 bp, synthetic construct
  misc_feature 1..22: note = Synthetic construct
  source 1..22: mol_type = other DNA
ttccctttctgcttcatcttgc

SEQ ID NO: 5 - DNA, 19 bp, synthetic construct
  misc_feature 1..19: note = Synthetic construct
  source 1..19: mol_type = other DNA
gaagcagcacgacttcttc

SEQ ID NO: 6 - DNA, 21 bp, synthetic construct
  misc_feature 1..21: note = Synthetic construct
  source 1..21: mol_type = other DNA
cctgagacagatcagcaacaa

SEQ ID NO: 7 - DNA, 20 bp, synthetic construct
  misc_feature 1..20: note = Synthetic construct
  source 1..20: mol_type = other DNA
cctaccctctcaacgacagc

SEQ ID NO: 8 - DNA, 20 bp, synthetic construct
  misc_feature 1..20: note = Synthetic construct
  source 1..20: mol_type = other DNA
ctctgaccttttgccaggag

SEQ ID NO: 9 - DNA, 20 bp, synthetic construct
  misc_feature 1..20: note = Synthetic construct
  source 1..20: mol_type = other DNA
cgacttcaccaactggttct

SEQ ID NO: 10 - DNA, 19 bp, synthetic construct
  misc_feature 1..19: note = Synthetic construct
  source 1..19: mol_type = other DNA
ccgtgaatgattggagtgc

SEQ ID NO: 11 - DNA, 19 bp, synthetic construct
  misc_feature 1..19: note = Synthetic construct
  source 1..19: mol_type = other DNA
gctctgccaagatggagag

SEQ ID NO: 12 - DNA, 19 bp, synthetic construct
  misc_feature 1..19: note = Synthetic construct
  source 1..19: mol_type = other DNA
ctgtcgcttgacttgcttg

SEQ ID NO: 13 - DNA, 20 bp, synthetic construct
  misc_feature 1..20: note = Synthetic construct
  source 1..20: mol_type = other DNA
acctcgggactcaacacctc

SEQ ID NO: 14 - DNA, 18 bp, synthetic construct
  misc_feature 1..18: note = Synthetic construct
  source 1..18: mol_type = other DNA
ctgaggcccgtaggaatc

SEQ ID NO: 15 - DNA, 19 bp, synthetic construct
  misc_feature 1..19: note = Synthetic construct
  source 1..19: mol_type = other DNA
ctccttctccaatcagatg

SEQ ID NO: 16 - DNA, 19 bp, synthetic construct
  misc_feature 1..19: note = Synthetic construct
  source 1..19: mol_type = other DNA
caagactgggcacctagtg

SEQ ID NO: 17 - DNA, 20 bp, synthetic construct
  misc_feature 1..20: note = Synthetic construct
  source 1..20: mol_type = other DNA
gtgtggttacaggcgaggat

SEQ ID NO: 18 - DNA, 20 bp, synthetic construct
  misc_feature 1..20: note = Synthetic construct
  source 1..20: mol_type = other DNA
gatgacatctcggcctttgt

SEQ ID NO: 19 - DNA, 19 bp, synthetic construct
  misc_feature 1..19: note = Synthetic construct
  source 1..19: mol_type = other DNA
gtcttcccctccatcgtgg

SEQ ID NO: 20 - DNA, 20 bp, synthetic construct
  misc_feature 1..20: note = Synthetic construct
  source 1..20: mol_type = other DNA
gatgcctctcttgctctggg

SEQ ID NO: 21 - DNA, 20 bp, synthetic construct
  misc_feature 1..20: note = Synthetic construct
  source 1..20: mol_type = other DNA
acggcactcctagtctggaa

SEQ ID NO: 22 - DNA, 21 bp, synthetic construct
  misc_feature 1..21: note = Synthetic construct
  source 1..21: mol_type = other DNA
ccacgtcaatctcttcacctt

SEQ ID NO: 23 - DNA, 20 bp, synthetic construct
  misc_feature 1..20: note = Synthetic construct
  source 1..20: mol_type = other DNA
cctagtgctgcatgaggaga

SEQ ID NO: 24 - DNA, 23 bp, synthetic construct
  misc_feature 1..23: note = Synthetic construct
  source 1..23: mol_type = other DNA
tcttcctcatcttcttgctcttc

SEQ ID NO: 25 - DNA, 24 bp, synthetic construct
  misc_feature 1..24: note = Synthetic construct
  source 1..24: mol_type = other DNA
ggcatagaggtctttacggatgtc

SEQ ID NO: 26 - DNA, 20 bp, synthetic construct
  misc_feature 1..20: note = Synthetic construct
  source 1..20: mol_type = other DNA
tattggcaacgagcggttcc

SEQ ID NO: 27 - protein, 439 aa, synthetic construct
  REGION 1..439: note = Synthetic construct
MPLNVNFTNRNYDLDYDSVQPYFICDEEENFYHQQQQSELQPPAPSEDIWKKFELLPAPPLSPSRRSGLCSPSYVAVATSFSPREDDDGGGGNFSTADQLEMMTELLGGDMVNQSFICDPDDETFIKNIIIQDCMWSGFSAAAKLVSEKLASYQAARKDSTSLSPARGHSVCSTSSLYLQDLTAAASECIDPSVVFPYPLNDSSSPKSCTSSDSTAFSPSSDSLLSSESSPRASPEPLVLHEETPPTTSSDSEEEQEDEEEIDVVSVEKRQTPAKRSESGSSPSRGHSKPPHSPLVLKRCHVSTHQHNYAAPPSTRKDYPAAKRAKLDSGRVLKQISNNRKCSSPRSSDTEENDKRRTHNVLERQRRNELKRSFFALRDQIPELENNEKAPKVVILKKATAYILSIQADEHKLTSEKDLLRKRREQLKHKLEQLRNSGA